European Patent Application EP 4 685 276 A1, published January 28, 2026. Title: METHOD FOR SIX-LETTER DNA APTAMER GENERATION. Applicant: Xenolis Pte. Ltd. Application JP. The sequence listing filed with the application follows.

SEQUENCE LISTING (242 sequences)

SEQ ID NO: 1 - DNA, 52 bp, synthetic construct
  source 1..52: mol_type = other DNA
  modified_base order(22,28,34): mod_base = OTHER; note = an unnatural base
ctccgcagtctgtggtgggacngggctnatgtangggatctgacaagcggag

SEQ ID NO: 2 - DNA, 31 bp, synthetic construct
  source 1..31: mol_type = other DNA
  modified_base order(12,18,24): mod_base = OTHER; note = an unnatural base
tgtggtgggacngggctnatgtangggatct

SEQ ID NO: 3 - DNA, 49 bp, synthetic construct
  source 1..49: mol_type = other DNA
  modified_base order(21,27,33): mod_base = OTHER; note = an unnatural base
ctccgcgtctgtggtgggacngggctnatgtangggatctgacgcggag

SEQ ID NO: 4 - DNA, 49 bp, synthetic construct
  source 1..49: mol_type = other DNA
  modified_base order(27,33): mod_base = OTHER; note = an unnatural base
ctccgcgtctgtggtgggactgggctnatgtangggatctgacgcggag

SEQ ID NO: 5 - DNA, 31 bp, synthetic construct
  source 1..31: mol_type = other DNA
  modified_base order(18,24): mod_base = OTHER; note = an unnatural base
tgtggtgggactgggctnatgtangggatct

SEQ ID NO: 6 - DNA, 49 bp, synthetic construct
  source 1..49: mol_type = other DNA
  modified_base order(21,33): mod_base = OTHER; note = an unnatural base
ctccgcgtctgtggtgggacngggctaatgtangggatctgacgcggag

SEQ ID NO: 7 - DNA, 31 bp, synthetic construct
  source 1..31: mol_type = other DNA
  modified_base order(12,24): mod_base = OTHER; note = an unnatural base
tgtggtgggacngggctaatgtangggatct

SEQ ID NO: 8 - DNA, 54 bp, synthetic construct
  source 1..54: mol_type = other DNA
  modified_base order(24,37): mod_base = OTHER; note = an unnatural base
gtcctcacgccgtcataattgttnttttgatccttgnagtggggacgtgaggac

SEQ ID NO: 9 - DNA, 36 bp, synthetic construct
  source 1..36: mol_type = other DNA
  modified_base order(15,28): mod_base = OTHER; note = an unnatural base
ccgtcataattgttnttttgatccttgnagtgggga

SEQ ID NO: 10 - DNA, 54 bp, synthetic construct
  source 1..54: mol_type = other DNA
  modified_base order(17,24,37): mod_base = OTHER; note = an unnatural base
gtcctcacgccgtcatnattgttnttttgatccttgnagtggggacgtgaggac

SEQ ID NO: 11 - DNA, 36 bp, synthetic construct
  source 1..36: mol_type = other DNA
  modified_base order(8,15,28): mod_base = OTHER; note = an unnatural base
ccgtcatnattgttnttttgatccttgnagtgggga

SEQ ID NO: 12 - DNA, 54 bp, synthetic construct
  source 1..54: mol_type = other DNA
  modified_base order(18,24,37): mod_base = OTHER; note = an unnatural base
gtcctcacgccgtcatanttgttnttttgatccttgnagtggggacgtgaggac

SEQ ID NO: 13 - DNA, 36 bp, synthetic construct
  source 1..36: mol_type = other DNA
  modified_base order(9,15,28): mod_base = OTHER; note = an unnatural base
ccgtcatanttgttnttttgatccttgnagtgggga

SEQ ID NO: 14 - DNA, 54 bp, synthetic construct; identical to SEQ ID NO: 10
  source 1..54: mol_type = other DNA
  modified_base order(17,24,37): mod_base = OTHER; note = an unnatural base

SEQ ID NO: 15 - DNA, 36 bp, synthetic construct; identical to SEQ ID NO: 11
  source 1..36: mol_type = other DNA
  modified_base order(8,15,28): mod_base = OTHER; note = an unnatural base

SEQ ID NO: 16 - DNA, 54 bp, synthetic construct; identical to SEQ ID NO: 12
  source 1..54: mol_type = other DNA
  modified_base order(18,24,37): mod_base = OTHER; note = an unnatural base

SEQ ID NO: 17 - DNA, 36 bp, synthetic construct; identical to SEQ ID NO: 13
  source 1..36: mol_type = other DNA
  modified_base order(9,15,28): mod_base = OTHER; note = an unnatural base

SEQ ID NO: 18 - DNA, 54 bp, synthetic construct
  source 1..54: mol_type = other DNA
  modified_base order(17,18,24,37): mod_base = OTHER; note = an unnatural base
gtcctcacgccgtcatnnttgttnttttgatccttgnagtggggacgtgaggac

SEQ ID NO: 19 - DNA, 36 bp, synthetic construct
  source 1..36: mol_type = other DNA
  modified_base order(8,9,15,28): mod_base = OTHER; note = an unnatural base
ccgtcatnnttgttnttttgatccttgnagtgggga

SEQ ID NO: 20 - DNA, 51 bp, synthetic construct
  source 1..51: mol_type = other DNA
  modified_base order(9,20,32): mod_base = OTHER; note = an unnatural base
gctgcttcngccatgacccntttcagccggcntggtcatgtgacaagcagc

SEQ ID NO: 21 - DNA, 15 bp, synthetic construct
  source 1..15: mol_type = other DNA
  modified_base order(2,14): mod_base = OTHER; note = an unnatural base
cntttcagccggcnt

SEQ ID NO: 22 - DNA, 51 bp, synthetic construct
  source 1..51: mol_type = other DNA
  modified_base order(20,32): mod_base = OTHER; note = an unnatural base
gctgcttcagccatgacccntttcagccggcntggtcatgtgacaagcagc

SEQ ID NO: 23 - DNA, 50 bp, synthetic construct
  source 1..50: mol_type = other DNA
  modified_base order(9,20,31): mod_base = OTHER; note = an unnatural base
gctgcttcngccatgacccnttcagccggcntggtcatgtgacaagcagc

SEQ ID NO: 24 - DNA, 14 bp, synthetic construct
  source 1..14: mol_type = other DNA
  modified_base order(2,13): mod_base = OTHER; note = an unnatural base
cnttcagccggcnt

SEQ ID NO: 25 - DNA, 39 bp, synthetic construct
  source 1..39: mol_type = other DNA
  modified_base order(14,26): mod_base = OTHER; note = an unnatural base
cgctgcatgacccntttcagccggcntggtcatgcagcg

SEQ ID NO: 26 - DNA, 38 bp, synthetic construct
  source 1..38: mol_type = other DNA
  modified_base order(14,25): mod_base = OTHER; note = an unnatural base
cgctgcatgacccnttcagccggcntggtcatgcagcg

SEQ ID NO: 27 - DNA, 48 bp, synthetic construct
  source 1..48: mol_type = other DNA
  modified_base order(16,22): mod_base = OTHER; note = an unnatural base
gtcacgcgctgtggtngttttnttgggggggtggttaaggcgcgtgac

SEQ ID NO: 28 - DNA, 28 bp, synthetic construct
  source 1..28: mol_type = other DNA
  modified_base order(6,12): mod_base = OTHER; note = an unnatural base
gtggtngttttnttgggggggtggttaa

SEQ ID NO: 29 - DNA, 43 bp, synthetic construct
  source 1..43: mol_type = other DNA
  modified_base order(10,16,28): mod_base = OTHER; note = an unnatural base
gcacgctttnacttantggctgggtggnctgggtaaagcgtgc

SEQ ID NO: 30 - DNA, 25 bp, synthetic construct
  source 1..25: mol_type = other DNA
  modified_base order(1,7,19): mod_base = OTHER; note = an unnatural base
nacttantggctgggtggnctgggt

SEQ ID NO: 31 - DNA, 53 bp, synthetic construct
  source 1..53: mol_type = other DNA
  modified_base order(26,41): mod_base = OTHER; note = an unnatural base
gctgtcacgcagcatggaacctttantggctaggggtgggnggaggtgacagc

SEQ ID NO: 32 - DNA, 37 bp, synthetic construct
  source 1..37: mol_type = other DNA
  modified_base order(18,33): mod_base = OTHER; note = an unnatural base
gcagcatggaacctttantggctaggggtgggnggag

SEQ ID NO: 33 - DNA, 51 bp, synthetic construct
  source 1..51: mol_type = other DNA
  modified_base order(16,24,35): mod_base = OTHER; note = an unnatural base
gcgttgcgtgaagttngggtgggnatgtgatgggnggtagatagacaacgc

SEQ ID NO: 34 - DNA, 39 bp, synthetic construct
  source 1..39: mol_type = other DNA
  modified_base order(10,18,29): mod_base = OTHER; note = an unnatural base
cgtgaagttngggtgggnatgtgatgggnggtagataga

SEQ ID NO: 35 - DNA, 51 bp, synthetic construct
  source 1..51: mol_type = other DNA
  modified_base order(17,24,36,39): mod_base = OTHER; note = an unnatural base
gctgatctcggaagganggtgggntctgggttgggnggngcgtagatcagc

SEQ ID NO: 36 - DNA, 35 bp, synthetic construct
  source 1..35: mol_type = other DNA
  modified_base order(9,16,28,31): mod_base = OTHER; note = an unnatural base
cggaagganggtgggntctgggttgggnggngcgt

SEQ ID NO: 37 - DNA, 46 bp, synthetic construct
  source 1..46: mol_type = other DNA
  modified_base order(29,38): mod_base = OTHER; note = an unnatural base
gcacgaggcagggttgggagggtaagganggtgggtgncctcgtgc

SEQ ID NO: 38 - DNA, 25 bp, synthetic construct
  source 1..25: mol_type = other DNA
  modified_base 19: mod_base = OTHER; note = an unnatural base
gggttgggagggtaagganggtggg

SEQ ID NO: 39 - DNA, 43 bp, synthetic construct
  source 1..43: mol_type = other DNA
  modified_base order(13,20,25,34): mod_base = OTHER; note = an unnatural base
gcacgtggggtcnccgatgnccatnaccacaggnaccacgtgc

SEQ ID NO: 40 - DNA, 23 bp, synthetic construct
  source 1..23: mol_type = other DNA
  modified_base order(2,9,14,23): mod_base = OTHER; note = an unnatural base
cnccgatgnccatnaccacaggn

SEQ ID NO: 41 - DNA, 57 bp, synthetic construct
  source 1..57: mol_type = other DNA
  modified_base order(17,33,38): mod_base = OTHER; note = an unnatural base
gctccgcgccgtacacnagtccgctagacatgncagtnacgagtggacaagcggagc

SEQ ID NO: 42 - DNA, 26 bp, synthetic construct
  source 1..26: mol_type = other DNA
  modified_base order(1,17,22): mod_base = OTHER; note = an unnatural base
nagtccgctagacatgncagtnacga

SEQ ID NO: 43 - DNA, 45 bp, synthetic construct
  source 1..45: mol_type = other DNA
  modified_base order(17,26): mod_base = OTHER; note = an unnatural base
ggagatgctaactcaanccggtggcnaggcgagttgaacatctcc

SEQ ID NO: 44 - DNA, 16 bp, synthetic construct
  source 1..16: mol_type = other DNA
  modified_base order(3,12): mod_base = OTHER; note = an unnatural base
aanccggtggcnaggc

SEQ ID NO: 45 - DNA, 45 bp, synthetic construct
  source 1..45: mol_type = other DNA
  modified_base order(17,26): mod_base = OTHER; note = an unnatural base
gactccgcttgaacaanccggtgggnaggcgtgacaagcggagtc

SEQ ID NO: 46 - DNA, 16 bp, synthetic construct
  source 1..16: mol_type = other DNA
  modified_base order(3,12): mod_base = OTHER; note = an unnatural base
aanccggtgggnaggc

SEQ ID NO: 47 - DNA, 45 bp, synthetic construct
  source 1..45: mol_type = other DNA
  modified_base order(17,26,37): mod_base = OTHER; note = an unnatural base
ggagatgctaactcaanccggtggcnaggcgagttgnacatctcc

SEQ ID NO: 48 - DNA, 42 bp, synthetic construct
  source 1..42: mol_type = other DNA
  modified_base order(16,25): mod_base = OTHER; note = an unnatural base
gactccgcttgacaanccggtgggnaggcgtcaagcggagtc

SEQ ID NO: 49 - DNA, 50 bp, synthetic construct
  source 1..50: mol_type = other DNA
  modified_base order(17,23,30): mod_base = OTHER; note = an unnatural base
gttcacgagagtgtgcnccatancacgggnaggtgacatatatcgtgaac

SEQ ID NO: 50 - DNA, 21 bp, synthetic construct
  source 1..21: mol_type = other DNA
  modified_base order(3,9,16): mod_base = OTHER; note = an unnatural base
gcnccatancacgggnaggtg

SEQ ID NO: 51 - DNA, 10 bp, synthetic construct
  source 1..10: mol_type = other DNA
ctccgcagtc

SEQ ID NO: 52 - DNA, 11 bp, synthetic construct
  source 1..11: mol_type = other DNA
gacaagcggag

SEQ ID NO: 53-56 - skipped (4 entries)

SEQ ID NO: 57 - DNA, 18 bp, synthetic construct
  source 1..18: mol_type = other DNA
  modified_base 9: mod_base = OTHER; note = an unnatural base
gctgcttcngccatgacc

SEQ ID NO: 58 - DNA, 18 bp, synthetic construct
  source 1..18: mol_type = other DNA
ggtcatgtgacaagcagc

SEQ ID NO: 59 - DNA, 18 bp, synthetic construct
  source 1..18: mol_type = other DNA
gctgcttcagccatgacc

SEQ ID NO: 60 - skipped

SEQ ID NO: 61 - DNA, 12 bp, synthetic construct
  source 1..12: mol_type = other DNA
cgctgcatgacc

SEQ ID NO: 62 - DNA, 12 bp, synthetic construct
  source 1..12: mol_type = other DNA
ggtcatgcagcg

SEQ ID NO: 63 - DNA, 10 bp, synthetic construct
  source 1..10: mol_type = other DNA
gtcacgcgct

SEQ ID NO: 64 - DNA, 10 bp, synthetic construct
  source 1..10: mol_type = other DNA
ggcgcgtgac

SEQ ID NO: 65-72 - skipped (8 entries)

SEQ ID NO: 73 - DNA, 10 bp, synthetic construct
  source 1..10: mol_type = other DNA
gcacgaggca

SEQ ID NO: 74 - DNA, 11 bp, synthetic construct
  source 1..11: mol_type = other DNA
  modified_base 3: mod_base = OTHER; note = an unnatural base
tgncctcgtgc

SEQ ID NO: 75 - DNA, 11 bp, synthetic construct
  source 1..11: mol_type = other DNA
gcacgtggggt

SEQ ID NO: 76 - skipped

SEQ ID NO: 77 - DNA, 16 bp, synthetic construct
  source 1..16: mol_type = other DNA
gctccgcgccgtacac

SEQ ID NO: 78 - DNA, 15 bp, synthetic construct
  source 1..15: mol_type = other DNA
gtggacaagcggagc

SEQ ID NO: 79 - DNA, 14 bp, synthetic construct
  source 1..14: mol_type = other DNA
ggagatgctaactc

SEQ ID NO: 80 - DNA, 15 bp, synthetic construct
  source 1..15: mol_type = other DNA
gagttgaacatctcc

SEQ ID NO: 81 - DNA, 14 bp, synthetic construct
  source 1..14: mol_type = other DNA
gactccgcttgaac

SEQ ID NO: 82 - DNA, 15 bp, synthetic construct
  source 1..15: mol_type = other DNA
gtgacaagcggagtc

SEQ ID NO: 83 - DNA, 15 bp, synthetic construct
  source 1..15: mol_type = other DNA
  modified_base 7: mod_base = OTHER; note = an unnatural base
gagttgnacatctcc

SEQ ID NO: 84 - DNA, 13 bp, synthetic construct
  source 1..13: mol_type = other DNA
gactccgcttgac

SEQ ID NO: 85 - DNA, 13 bp, synthetic construct
  source 1..13: mol_type = other DNA
gtcaagcggagtc

SEQ ID NO: 86 - DNA, 14 bp, synthetic construct
  source 1..14: mol_type = other DNA
gttcacgagagtgt

SEQ ID NO: 87 - DNA, 15 bp, synthetic construct
  source 1..15: mol_type = other DNA
acatatatcgtgaac

SEQ ID NO: 88 - DNA, 72 bp, synthetic construct
  source 1..72: mol_type = other DNA
  modified_base order(11,23,35): mod_base = OTHER; note = an unnatural base
ggctggtccgnctgggaacaagnggcgggagggangggtgtgggtgcgacaagcggaccagggcgcgtagcg

SEQ ID NO: 89 - DNA, 58 bp, synthetic construct
  source 1..58: mol_type = other DNA
  modified_base order(25,31,37): mod_base = OTHER; note = an unnatural base
ctgctccgcagtctgtggtgggacngggctnatgtangggatctgacaagcggagtag

SEQ ID NO: 90 - DNA, 64 bp, synthetic construct
  source 1..64: mol_type = other DNA
  modified_base order(26,37,51): mod_base = OTHER; note = an unnatural base
tgattagctgagacctgatgctgtgnctgggtggggnccttagcgtttggncatcggctgaagg

SEQ ID NO: 91 - DNA, 64 bp, synthetic construct
  source 1..64: mol_type = other DNA
  modified_base order(19,29,39,46): mod_base = OTHER; note = an unnatural base
agacctgatgctggggcgnggggtgggantgtgtgggcncgggggncctgataagacaagcgga

SEQ ID NO: 92 - DNA, 47 bp, synthetic construct
  source 1..47: mol_type = other DNA
  modified_base order(17,26,36): mod_base = OTHER; note = an unnatural base
atgctagatacgcagcnttagtcaanggaattgcgngtataagggtt

SEQ ID NO: 93 - DNA, 55 bp, synthetic construct
  source 1..55: mol_type = other DNA
  modified_base order(34,37): mod_base = OTHER; note = an unnatural base
attctcacgccgtcataattgttnttttgatccttgnagtggggacgtgacaagc

SEQ ID NO: 94 - DNA, 55 bp, synthetic construct
  source 1..55: mol_type = other DNA
  modified_base order(13,19,29,34,41): mod_base = OTHER; note = an unnatural base
attctcacgtaanggtatnggatttgcgnggggnagggttnccaacgtgacaagc

SEQ ID NO: 95 - DNA, 55 bp, synthetic construct
  source 1..55: mol_type = other DNA
  modified_base order(29,42): mod_base = OTHER; note = an unnatural base
attctcacgcaagacctctcgggagagtntacgaagttgtanttgcgtgacaagc

SEQ ID NO: 96 - DNA, 55 bp, synthetic construct
  source 1..55: mol_type = other DNA
  modified_base order(19,25,31): mod_base = OTHER; note = an unnatural base
attctcacgtcgcggaaanggtatngtacgncgttggtttcccggcgtgacaagc

SEQ ID NO: 97 - DNA, 55 bp, synthetic construct
  source 1..55: mol_type = other DNA
  modified_base order(14,36): mod_base = OTHER; note = an unnatural base
attctcacgagatngctaacgacggggctttaggcnaatttacctcgtgacaagc

SEQ ID NO: 98 - DNA, 60 bp, synthetic construct
  source 1..60: mol_type = other DNA
  modified_base order(14,25,37): mod_base = OTHER; note = an unnatural base
tgcttgcggcttcngccatgacccntttcagccggcntggtcatgtgacaagcggagtag

SEQ ID NO: 99 - DNA, 60 bp, synthetic construct
  source 1..60: mol_type = other DNA
  modified_base order(25,37,50): mod_base = OTHER; note = an unnatural base
agctgagacctgatgctgcgaaccntttcagccggcntgttcgagcagcncttccaaggg

SEQ ID NO: 100 - DNA, 60 bp, synthetic construct
  source 1..60: mol_type = other DNA
  modified_base order(19,25,37): mod_base = OTHER; note = an unnatural base
tgctactccatagataacnctaccntttcagccggcntgtatgttagacaagcggagtag

SEQ ID NO: 101 - DNA, 59 bp, synthetic construct
  source 1..59: mol_type = other DNA
  modified_base order(19,25,36): mod_base = OTHER; note = an unnatural base
tgcttacggaccaattggntggccnttcagccggcntgccaccaacgacaagcggagta

SEQ ID NO: 102 - DNA, 60 bp, synthetic construct
  source 1..60: mol_type = other DNA
  modified_base order(13,25,37): mod_base = OTHER; note = an unnatural base
atgctatacgttngccactgggccntttcagccggcntgcccaggtggacaagcggagta

SEQ ID NO: 103 - DNA, 59 bp, synthetic construct
  source 1..59: mol_type = other DNA
  modified_base order(16,25,36,42): mod_base = OTHER; note = an unnatural base
ctgatgcttgggcatnggagcaccnttcagccggcntgtgcngccgccgtgacaagcgg

SEQ ID NO: 104 - DNA, 60 bp, synthetic construct
  source 1..60: mol_type = other DNA
  modified_base order(30,45): mod_base = OTHER; note = an unnatural base
cctgatgctcacgcagcatggaacctttantggctaggggtgggnggaggtgacaagcgg

SEQ ID NO: 105 - DNA, 54 bp, synthetic construct
  source 1..54: mol_type = other DNA
  modified_base order(24,33): mod_base = OTHER; note = an unnatural base
tgctgatcccgccgcgcagattantggtttganatagggtggttaggacaagcg

SEQ ID NO: 106 - DNA, 55 bp, synthetic construct
  source 1..55: mol_type = other DNA
  modified_base order(16,24,33,38): mod_base = OTHER; note = an unnatural base
tgctttcggcctatgnagcgcgcnagggtgggntcttgntggttgggacaagcgt

SEQ ID NO: 107 - DNA, 53 bp, synthetic construct
  source 1..53: mol_type = other DNA
  modified_base order(17,25,36): mod_base = OTHER; note = an unnatural base
ctggttgcgtgaagttngggtgggnatgtgatgggnggtagatagacaagcgg

SEQ ID NO: 108 - DNA, 54 bp, synthetic construct
  source 1..54: mol_type = other DNA
  modified_base order(37,40): mod_base = OTHER; note = an unnatural base
tgcttatcttacaagcgcggatcttantggttggggtggntttggggacaagcg

SEQ ID NO: 109 - DNA, 65 bp, synthetic construct
  source 1..65: mol_type = other DNA
  modified_base order(25,32,44,47): mod_base = OTHER; note = an unnatural base
gctgagacctgatgctcggaagganggtgggntctgggttgggnggngcgtagatcaggacaagc

SEQ ID NO: 110 - DNA, 64 bp, synthetic construct
  source 1..64: mol_type = other DNA
  modified_base order(38,47): mod_base = OTHER; note = an unnatural base
ctcctattctcacgaggcagggttgggagggtaagganggtgggtgncctcgtgacaagcggag

SEQ ID NO: 111 - DNA, 64 bp, synthetic construct
  source 1..64: mol_type = other DNA
  modified_base order(29,35,45): mod_base = OTHER; note = an unnatural base
ctcctattctcacggcaaacgcactttantggtgngggtgggctngtcttcgtgacaagcggag

SEQ ID NO: 112 - DNA, 64 bp, synthetic construct
  source 1..64: mol_type = other DNA
  modified_base order(19,31,36): mod_base = OTHER; note = an unnatural base
ctcctattctcacgtagcnggtccgggttantgggngggtggcttggggccgtgacaagcggag

SEQ ID NO: 113 - DNA, 64 bp, synthetic construct
  source 1..64: mol_type = other DNA
  modified_base order(24,30): mod_base = OTHER; note = an unnatural base
ctcctattctcacgcgctgtggtngttttnttgggggggtggttaaggcgcgtgacaagcggag

SEQ ID NO: 114 - DNA, 64 bp, synthetic construct
  source 1..64: mol_type = other DNA
  modified_base order(19,25,37): mod_base = OTHER; note = an unnatural base
ctcctattctcacgctttnacttantggctgggtggnctgggtaaagacgcgtgacaagcggaa

SEQ ID NO: 115 - DNA, 61 bp, synthetic construct
  source 1..61: mol_type = other DNA
  modified_base order(19,35,40): mod_base = OTHER; note = an unnatural base
atgctccgcgccgtacacnagtccgctagacatgncagtnacgagtggacaagcggagtag

SEQ ID NO: 116 - DNA, 61 bp, synthetic construct
  source 1..61: mol_type = other DNA
  modified_base order(13,22,29): mod_base = OTHER; note = an unnatural base
atgcttggctganctgacaaancaggggnccccgtaaactgtgtcacgacaagcggagtag

SEQ ID NO: 117 - DNA, 61 bp, synthetic construct
  source 1..61: mol_type = other DNA
  modified_base order(13,25,32): mod_base = OTHER; note = an unnatural base
atgcttggtaggntactactctagnggagatntgggccgggtttgtcgacaagcggagtag

SEQ ID NO: 118 - DNA, 66 bp, synthetic construct
  source 1..66: mol_type = other DNA
  modified_base order(23,30,35,44): mod_base = OTHER; note = an unnatural base
tctcctattctcacgtggggtcnccgatgnccatnaccacaggnaccacatcgtgacaagcggagt

SEQ ID NO: 119 - DNA, 66 bp, synthetic construct
  source 1..66: mol_type = other DNA
  modified_base order(22,25,32,41,46): mod_base = OTHER; note = an unnatural base
tctcctattctcacgggcgatncancaggtgnccacaattnccggnatttccgtgacaagcggagt

SEQ ID NO: 120 - DNA, 66 bp, synthetic construct
  source 1..66: mol_type = other DNA
  modified_base order(25,35,41): mod_base = OTHER; note = an unnatural base
tctcctattctcacggccgcacccngctccttcgncaatcncggcctcggccgtgacaagcggagt

SEQ ID NO: 121 - DNA, 66 bp, synthetic construct
  source 1..66: mol_type = other DNA
  modified_base order(23,38,44,48): mod_base = OTHER; note = an unnatural base
tctcctattctcacgaaattaanctcagctagaattgncccccncagnaatcgtgacaagcggagt

SEQ ID NO: 122 - DNA, 66 bp, synthetic construct
  source 1..66: mol_type = other DNA
  modified_base order(28,35,48): mod_base = OTHER; note = an unnatural base
tctcctattctcacgctcaaatgtttcnccggggnaccatctacaggntaacgtgacaagcggagt

SEQ ID NO: 123 - DNA, 54 bp, synthetic construct
  source 1..54: mol_type = other DNA
  modified_base order(19,28,43): mod_base = OTHER; note = an unnatural base
tgatgcttgattgcccaanccgttggcnaggcgggcaataccngaataagacaa

SEQ ID NO: 124 - DNA, 54 bp, synthetic construct
  source 1..54: mol_type = other DNA
  modified_base order(19,28,39): mod_base = OTHER; note = an unnatural base
gacctgatgctaactcaanccggtggcnaggcgagttgnacatcttctatcagg

SEQ ID NO: 125 - DNA, 54 bp, synthetic construct
  source 1..54: mol_type = other DNA
  modified_base order(19,28): mod_base = OTHER; note = an unnatural base
gacctgatgctcgactaanccggtgggnaggcacggagaagcatgggtttctag

SEQ ID NO: 126 - DNA, 54 bp, synthetic construct
  source 1..54: mol_type = other DNA
  modified_base order(19,31,37): mod_base = OTHER; note = an unnatural base
tgcttgtgaaagtggggcnctcgccggaggnagtggnaacgttaaagacaagcg

SEQ ID NO: 127 - DNA, 54 bp, synthetic construct
  source 1..54: mol_type = other DNA
  modified_base order(10,24,33): mod_base = OTHER; note = an unnatural base
aaggcttacngagcttaacccaanccggtggcnaggcggggacaagcggagtag

SEQ ID NO: 128 - DNA, 56 bp, synthetic construct
  source 1..56: mol_type = other DNA
  modified_base order(21,27,34): mod_base = OTHER; note = an unnatural base
ctattctcacgagagtgtgcnccatancacgggnaggtgacatatatcgtgacaag

SEQ ID NO: 129 - DNA, 56 bp, synthetic construct
  source 1..56: mol_type = other DNA
  modified_base order(9,15,23,32): mod_base = OTHER; note = an unnatural base
gactaacanatcgcnggagcaanccgttggcnaggcgtgacaagcggagtagttag

SEQ ID NO: 130 - DNA, 56 bp, synthetic construct
  source 1..56: mol_type = other DNA
  modified_base order(9,23,32): mod_base = OTHER; note = an unnatural base
cacgcgcgnttcatggtgccaanccggtggcnaggcggcccgtgacaagcggagta

SEQ ID NO: 131 - DNA, 56 bp, synthetic construct
  source 1..56: mol_type = other DNA
  modified_base order(14,20,26,35): mod_base = OTHER; note = an unnatural base
cacggccttgtccncccggngggggnaggggttanggttacgtgacaagcggagta

SEQ ID NO: 132 - DNA, 56 bp, synthetic construct
  source 1..56: mol_type = other DNA
  modified_base order(14,26,33): mod_base = OTHER; note = an unnatural base
tcacgcagacgccncccggcgggggnaggggantcgctcggcgtgacaagcggagt

SEQ ID NO: 133 - skipped

SEQ ID NO: 134 - DNA, 32 bp, synthetic construct
  source 1..32: mol_type = other DNA
  modified_base order(12,23): mod_base = OTHER; note = an unnatural base
gccaccgtatgnacgctcacagnagttgccga

SEQ ID NO: 135 - DNA, 52 bp, synthetic construct
  source 1..52: mol_type = other DNA
  modified_base order(22,33): mod_base = OTHER; note = an unnatural base
ctccttcagcgccaccgtatgnacgctcacagnagttgccgagctgaaggag

SEQ ID NO: 136 - DNA, 52 bp, synthetic construct
  source 1..52: mol_type = other DNA
ctccgcagtctgtggtgggactgggctaatgtaagggatctgacaagcggag

SEQ ID NO: 137 - DNA, 49 bp, synthetic construct
  source 1..49: mol_type = other DNA
  modified_base order(21,27): mod_base = OTHER; note = an unnatural base
ctccgcgtctgtggtgggacngggctnatgtaagggatctgacgcggag

SEQ ID NO: 138 - DNA, 58 bp, synthetic construct
  source 1..58: mol_type = other DNA
  modified_base order(21,27,33): mod_base = OTHER; note = an unnatural base
ctccgcgtctgtggtgggacngggctnatgtangggatctgacgcggagcgcgtagcg

SEQ ID NO: 139 - DNA, 48 bp, synthetic construct
  source 1..48: mol_type = other DNA
  modified_base order(28,39): mod_base = OTHER; note = an unnatural base
cccgcccgggtccgcgaagcggtaggtntgggctaggcngctggcggg

SEQ ID NO: 140 - DNA, 57 bp, synthetic construct
  source 1..57: mol_type = other DNA
  modified_base order(28,29): mod_base = OTHER; note = an unnatural base
cccgcccgggtccgcgaagcggtaggtntgggctaggcngctggcgggcgcgtagcg

SEQ ID NO: 141 - DNA, 54 bp, synthetic construct
  source 1..54: mol_type = other DNA
  modified_base order(13,24,37): mod_base = OTHER; note = an unnatural base
gtcctcacgccgncataattgttnttttgatccttgnagtggggacgtgaggac

SEQ ID NO: 142 - DNA, 54 bp, synthetic construct
  source 1..54: mol_type = other DNA
  modified_base order(24,31,37): mod_base = OTHER; note = an unnatural base
gtcctcacgccgtcataattgttnttttganccttgnagtggggacgtgaggac

SEQ ID NO: 143 - DNA, 54 bp, synthetic construct; identical to SEQ ID NO: 8
  source 1..54: mol_type = other DNA
  modified_base order(24,37): mod_base = OTHER; note = an unnatural base

SEQ ID NO: 144 - DNA, 54 bp, synthetic construct; identical to SEQ ID NO: 10
  source 1..54: mol_type = other DNA
  modified_base order(17,24,37): mod_base = OTHER; note = an unnatural base

SEQ ID NO: 145 - DNA, 54 bp, synthetic construct; identical to SEQ ID NO: 12
  source 1..54: mol_type = other DNA
  modified_base order(18,24,37): mod_base = OTHER; note = an unnatural base

SEQ ID NO: 146 - DNA, 63 bp, synthetic construct
  source 1..63: mol_type = other DNA
  modified_base order(24,37): mod_base = OTHER; note = an unnatural base
gtcctcacgccgtcataattgttnttttgatccttgnagtggggacgtgaggaccgcgtagcg

SEQ ID NO: 147 - DNA, 63 bp, synthetic construct
  source 1..63: mol_type = other DNA
  modified_base order(18,24,37): mod_base = OTHER; note = an unnatural base
gtcctcacgccgtcatanttgttnttttgatccttgnagtggggacgtgaggaccgcgtagcg

SEQ ID NO: 148 - DNA, 57 bp, synthetic construct; identical to SEQ ID NO: 140
  source 1..57: mol_type = other DNA
  modified_base order(28,39): mod_base = OTHER; note = an unnatural base

SEQ ID NO: 149 - DNA, 51 bp, synthetic construct; identical to SEQ ID NO: 20
  source 1..51: mol_type = other DNA
  modified_base order(9,20,32): mod_base = OTHER; note = an unnatural base

SEQ ID NO: 150 - DNA, 51 bp, synthetic construct
  source 1..51: mol_type = other DNA
  modified_base order(9,32): mod_base = OTHER; note = an unnatural base
gctgcttcngccatgacccatttcagccggcntggtcatgtgacaagcagc

SEQ ID NO: 151 - DNA, 51 bp, synthetic construct
  source 1..51: mol_type = other DNA
  modified_base order(9,20): mod_base = OTHER; note = an unnatural base
gctgcttcngccatgacccntttcagccggcttggtcatgtgacaagcagc

SEQ ID NO: 152 - DNA, 38 bp, synthetic construct; identical to SEQ ID NO: 26
  source 1..38: mol_type = other DNA
  modified_base order(14,25): mod_base = OTHER; note = an unnatural base

SEQ ID NO: 153 - DNA, 50 bp, synthetic construct
  source 1..50: mol_type = other DNA
  modified_base order(22,31): mod_base = OTHER; note = an unnatural base
gctgtcccgccgcgcagattantggtttganatagggtggttaggacagc

SEQ ID NO: 154 - DNA, 58 bp, synthetic construct
  source 1..58: mol_type = other DNA
  modified_base order(26,32,42): mod_base = OTHER; note = an unnatural base
gtccgttcacggcaaacgcactttantggtgngggtgggctngtcttcgtgaacggac

SEQ ID NO: 155 - DNA, 58 bp, synthetic construct
  source 1..58: mol_type = other DNA
  modified_base order(16,28,33): mod_base = OTHER; note = an unnatural base
gtcctttcacgtagcnggtccgggttantgggngggtggcttggggccgtgaaaggac

SEQ ID NO: 156 - DNA, 59 bp, synthetic construct
  source 1..59: mol_type = other DNA
  modified_base order(15,23,34): mod_base = OTHER; note = an unnatural base
gcgtgcgtgaagttngggtgggnatgtgatgggnggtagatacgcaacgccgcgtagcg

SEQ ID NO: 157 - DNA, 57 bp, synthetic construct
  source 1..57: mol_type = other DNA
  modified_base order(16,22): mod_base = OTHER; note = an unnatural base
gtcacgcgctgtggtngttttnttgggggggtggttaaggcgcgtgaccgcgtagcg

SEQ ID NO: 158 - DNA, 52 bp, synthetic construct
  source 1..52: mol_type = other DNA
  modified_base order(10,16,28): mod_base = OTHER; note = an unnatural base
gcacgctttnacttantggctgggtggnctgggtaaagcgtgccgcgtagcg

SEQ ID NO: 159 - DNA, 40 bp, synthetic construct
  source 1..40: mol_type = other DNA
gtgacgtaggttggtgtggttggggcgtcaccgcgtagcg

SEQ ID NO: 160 - DNA, 66 bp, synthetic construct
  source 1..66: mol_type = other DNA
gctccgcgccgtacacnagtccgctagacatgncagtnacgagtggacaagcggagccgcgtagcg

SEQ ID NO: 161 - DNA, 52 bp, synthetic construct
  source 1..52: mol_type = other DNA
  modified_base order(13,20,25,34): mod_base = OTHER; note = an unnatural base
gcacgtggggtcnccgatgnccatnaccacaggnaccacgtgccgcgtagcg

SEQ ID NO: 162 - DNA, 53 bp, synthetic construct
  source 1..53: mol_type = other DNA
  modified_base order(7,14,19,28): mod_base = OTHER; note = an unnatural base
gcggtcnccgatgnccatnaccacaggnaccacatcgtgaccgccgcgtagcg

SEQ ID NO: 163 - DNA, 44 bp, synthetic construct
  source 1..44: mol_type = other DNA
  modified_base order(9,14,23): mod_base = OTHER; note = an unnatural base
gtccgatgnccatnaccacaggnaccacatcggaccgcgtagcg

SEQ ID NO: 164 - DNA, 50 bp, synthetic construct; identical to SEQ ID NO: 49
  source 1..50: mol_type = other DNA
  modified_base order(17,23,30): mod_base = OTHER; note = an unnatural base

SEQ ID NO: 165 - DNA, 45 bp, synthetic construct; identical to SEQ ID NO: 43
  source 1..45: mol_type = other DNA
  modified_base order(17,26): mod_base = OTHER; note = an unnatural base

SEQ ID NO: 166 - DNA, 54 bp, synthetic construct
  source 1..54: mol_type = other DNA
  modified_base order(17,26): mod_base = OTHER; note = an unnatural base
ggagatgctaactcaanccggtggcnaggcgagttgaacatctcccgcgtagcg

SEQ ID NO: 167 - DNA, 54 bp, synthetic construct
  source 1..54: mol_type = other DNA
  modified_base order(17,26,37): mod_base = OTHER; note = an unnatural base
ggagatgctaactcaanccggtggcnaggcgagttgnacatctcccgcgtagcg

SEQ ID NO: 168 - DNA, 45 bp, synthetic construct; identical to SEQ ID NO: 45
  source 1..45: mol_type = other DNA
  modified_base order(17,26): mod_base = OTHER; note = an unnatural base

SEQ ID NO: 169 - DNA, 54 bp, synthetic construct
  source 1..54: mol_type = other DNA
  modified_base order(17,26): mod_base = OTHER; note = an unnatural base
gactccgcttgaacaanccggtgggnaggcgtgacaagcggagtccgcgtagcg

SEQ ID NO: 170 - DNA, 51 bp, synthetic construct
  source 1..51: mol_type = other DNA
  modified_base order(16,25): mod_base = OTHER; note = an unnatural base
gactccgcttgacaanccggtgggnaggcgtcaagcggagtccgcgtagcg

SEQ ID NO: 171 - DNA, 61 bp, synthetic construct
  source 1..61: mol_type = other DNA
  modified_base order(22,33): mod_base = OTHER; note = an unnatural base
ctccttcagcgccaccgtatgnacgctcacagnagttgccgagctgaaggagcgcgtagcg

SEQ ID NO: 172 - DNA, 61 bp, synthetic construct
  source 1..61: mol_type = other DNA
ctccttcagcgccaccgtatgaacgctcacagaagttgccgagctgaaggagcgcgtagcg

SEQ ID NO: 173 - DNA, 87 bp, synthetic construct
  source 1..87: mol_type = other DNA
  misc_difference 23..64: note = random sequence
tgattagctgagacctgatgctnnnnnnnnnnnnnnnnnnnnnnnnnnnnnnnnnnnnnnnnnngacaagcggagtagttagaccgt

SEQ ID NO: 174 - DNA, 94 bp, synthetic construct
  source 1..94: mol_type = other DNA
  misc_difference 27..68
gctcattcgcctctcctattctcacgnnnnnnnnnnnnnnnnnnnnnnnnnnnnnnnnnnnnnnnnnncgtgacaagcggagtagttagaccgt

SEQ ID NO: 175 - DNA, 58 bp, synthetic construct
  source 1..58: mol_type = other DNA
  modified_base order(22,28,38): mod_base = OTHER; note = an unnatural base
ctgatgctcctatgtcgctggnctgcanagtcgctggncaagggattagggacaagcg

SEQ ID NO: 176 - DNA, 58 bp, synthetic construct
  source 1..58: mol_type = other DNA
  modified_base order(15,29,39,44): mod_base = OTHER; note = an unnatural base
ctgatgctcgtgcgngtacgcggcgtggntggtgctggntgggncaggcggacaagcg

SEQ ID NO: 177 - DNA, 50 bp, synthetic construct
  source 1..50: mol_type = other DNA
  modified_base order(14,20,30): mod_base = OTHER; note = an unnatural base
cctatgtcgctggnctgcanagtcgctggncaagggattagggacaagcg

SEQ ID NO: 178 - DNA, 59 bp, synthetic construct
  source 1..59: mol_type = other DNA
  modified_base order(18,24,34): mod_base = OTHER; note = an unnatural base
ggctcctatgtcgctggnctgcanagtcgctggncaagggattaggagcccgcgtagcg

SEQ ID NO: 179 - DNA, 59 bp, synthetic construct
  source 1..59: mol_type = other DNA
  modified_base order(18,34): mod_base = OTHER; note = an unnatural base
ggctcctatgtcgctggnctgcatagtcgctggncaagggattaggagcccgcgtagcg

SEQ ID NO: 180 - DNA, 42 bp, synthetic construct
  source 1..42: mol_type = other DNA
  modified_base order(7,21,31): mod_base = OTHER; note = an unnatural base
cgtgcgngtacgcggcgtggntggtgctggntgggdcaggcg

SEQ ID NO: 181 - DNA, 58 bp, synthetic construct
  source 1..58: mol_type = other DNA
  modified_base order(10,24,34,39): mod_base = OTHER; note = an unnatural base
tgctccgcgngtacgcggcgtggntggtgctggntgggncaggcggacaagcggagca

SEQ ID NO: 182 - DNA, 67 bp, synthetic construct
  source 1..67: mol_type = other DNA
  modified_base order(10,24,34,39): mod_base = OTHER; note = an unnatural base
tgctccgcgngtacgcggcgtggntggtgctggntgggncaggcggacaagcggagcacgcgtagcg

SEQ ID NO: 183 - DNA, 67 bp, synthetic construct
  source 1..67: mol_type = other DNA
  modified_base order(24,34,39): mod_base = OTHER; note = an unnatural base
tgctccgcgtgtacgcggcgtggntggtgctggntgggncaggcggacaagcggagcacgcgtagcg

SEQ ID NO: 184 - DNA, 67 bp, synthetic construct; identical to SEQ ID NO: 183
  source 1..67: mol_type = other DNA
  modified_base order(24,34,39): mod_base = OTHER; note = an unnatural base

SEQ ID NO: 185 - DNA, 95 bp, synthetic construct
  source 1..95: mol_type = other DNA
  misc_difference order(23..31,58..72): note = random sequence
  modified_base order(40,44,46): mod_base = OTHER; note = an unnatural base
tgattagctgagacctgatgctnnnnnnnnngtcgctggnctgnanagtcgctggncnnnnnnnnnnnnnnngacaagcggagtagttagaccgt

SEQ ID NO: 186 - DNA, 67 bp, synthetic construct
  source 1..67: mol_type = other DNA
  modified_base order(20,26,36): mod_base = OTHER; note = an unnatural base
cttgtcaaggtgtcgctggnctgganagtcgctggncagaactttagccattgacaagcgcgtagcg

SEQ ID NO: 187 - DNA, 66 bp, synthetic construct
  source 1..66: mol_type = other DNA
  modified_base order(19,25,35): mod_base = OTHER; note = an unnatural base
cttgtcaggtgtcgctggnctgtanagtcgctggncagtacctttggccatgacaagcgcgtagcg

SEQ ID NO: 188 - DNA, 68 bp, synthetic construct
  source 1..68: mol_type = other DNA
  modified_base order(19,25,35): mod_base = OTHER; note = an unnatural base
ggcttgtcgtgtcgctggnctgaanagtcgctggncaaaaagctttttcgagacaagcccgcgtagcg

SEQ ID NO: 189 - DNA, 70 bp, synthetic construct
  source 1..70: mol_type = other DNA
  modified_base order(20,26,36): mod_base = OTHER; note = an unnatural base
ctgcttgtggtgtcgctggnctgcanagtcgctggncatgaaacctttggccgacaagcagcgcgtagcg

SEQ ID NO: 190 - DNA, 67 bp, synthetic construct
  source 1..67: mol_type = other DNA
  modified_base order(20,26,36): mod_base = OTHER; note = an unnatural base
cttgtcaaggagtcgctggnctgtanagtcgctggnctgtagtttacccattgacaagcgcgtagcg

SEQ ID NO: 191 - DNA, 58 bp, synthetic construct
  source 1..58: mol_type = other DNA
  modified_base order(20,26,36): mod_base = OTHER; note = an unnatural base
cttgtcaaggtgtcgctggnctgganagtcgctggncagaactttagccattgacaag

SEQ ID NO: 192 - DNA, 58 bp, synthetic construct
  source 1..58: mol_type = other DNA
  modified_base order(26,36): mod_base = OTHER; note = an unnatural base
cttgtcaaggtgtcgctggactgganagtcgctggncagaactttagccattgacaag

SEQ ID NO: 193 - DNA, 58 bp, synthetic construct
  source 1..58: mol_type = other DNA
  modified_base order(20,36): mod_base = OTHER; note = an unnatural base
cttgtcaaggtgtcgctggnctggatagtcgctggncagaactttagccattgacaag

SEQ ID NO: 194 - DNA, 58 bp, synthetic construct
  source 1..58: mol_type = other DNA
  modified_base order(20,26): mod_base = OTHER; note = an unnatural base
cttgtcaaggtgtcgctggnctgganagtcgctggacagaactttagccattgacaag

SEQ ID NO: 195 - DNA, 58 bp, synthetic construct
  source 1..58: mol_type = other DNA
cttgtcaaggtgtcgctggactggatagtcgctggacagaactttagccattgacaag

SEQ ID NO: 196 - DNA, 44 bp, synthetic construct
  source 1..44: mol_type = other DNA
  misc_difference order(22..24,37..44): note = random sequence
  modified_base order(18,34): mod_base = OTHER; note = an unnatural base
gtcccgcctgtcgctggnctgnnnagtcgctggncannnnnnnn

SEQ ID NO: 197 - DNA, 45 bp, synthetic construct
  source 1..45: mol_type = other DNA
  misc_difference order(22..24,37..45): note = random sequence
  modified_base order(18,34): mod_base = OTHER; note = an unnatural base
gtcccgcctgtcgctggnctgnnnagtcgctggncannnnnnnnn

SEQ ID NO: 198 - DNA, 46 bp, synthetic construct
  source 1..46: mol_type = other DNA
  misc_difference order(22..24,37..45): note = random sequence
  modified_base order(18,34): mod_base = OTHER; note = an unnatural base
gtcccgcctgtcgctggnctgnnnagtcgctggncannnnnnnnnn

SEQ ID NO: 199 - DNA, 65 bp, synthetic construct
  source 1..65: mol_type = other DNA
  modified_base order(19,25,35): mod_base = OTHER; note = an unnatural base
gggcccgcctgtcgctggnctgaanagtcgctggncaggtttccttcggcgggccccgcgtagcg

SEQ ID NO: 200 - DNA, 65 bp, synthetic construct
  source 1..65: mol_type = other DNA
  modified_base order(19,23,25,35): mod_base = OTHER; note = an unnatural base
gggcccgcctgtcgctggnctgnanagtcgctggncaggtttccttcggcgggccccgcgtagcg

SEQ ID NO: 201 - DNA, 65 bp, synthetic construct
  source 1..65: mol_type = other DNA
  modified_base order(19,25,35,41): mod_base = OTHER; note = an unnatural base
gggcccgcctgtcgctggnctgaanagtcgctggncaggtntccttcggcgggccccgcgtagcg

SEQ ID NO: 202 - DNA, 65 bp, synthetic construct
  source 1..65: mol_type = other DNA
  modified_base order(19,25,35,45): mod_base = OTHER; note = an unnatural base
gggcccgcctgtcgctggnctgaanagtcgctggncaggtttccntcggcgggccccgcgtagcg

SEQ ID NO: 203 - DNA, 65 bp, synthetic construct
  source 1..65: mol_type = other DNA
  modified_base order(19,25,35,41): mod_base = OTHER; note = an unnatural base
gggcccgcctgtcgctggnctgaanagtcgctggncaggtntccntcggcgggccccgcgtagcg

SEQ ID NO: 204 - DNA, 65 bp, synthetic construct
  source 1..65: mol_type = other DNA
  modified_base order(19,23,25,35): mod_base = OTHER; note = an unnatural base
gggcccgcctgtcgctggnctgnanagtcgctggncaggtntccntcggcgggccccgcgtagcg

SEQ ID NO: 205 - DNA, 63 bp, synthetic construct
  source 1..63: mol_type = other DNA
  modified_base order(19,25,35): mod_base = OTHER; note = an unnatural base
gggcccgcctgtcgctggnctgaanagtcgctggncaggtttccttccgggccccgcgtagcg

SEQ ID NO: 206 - DNA, 58 bp, synthetic construct
  source 1..58: mol_type = other DNA
  modified_base order(21,27,37): mod_base = OTHER; note = an unnatural base
gccgtcccgcctgtcgctggnctgaanagtcgctggncagcgggacggccgcgtagcg

SEQ ID NO: 207 - DNA, 58 bp, synthetic construct
  source 1..58: mol_type = other DNA
  modified_base order(21,27,37): mod_base = OTHER; note = an unnatural base
ggcggtcccgctgtcgctggnctgaanagtcgctggncacgggacggcccgcgtagcg

SEQ ID NO: 208 - DNA, 58 bp, synthetic construct
  source 1..58: mol_type = other DNA
  modified_base order(21,25,27,37): mod_base = OTHER; note = an unnatural base
ggcggtcccgctgtcgctggnctgnanagtcgctggncacgggacggcccgcgtagcg

SEQ ID NO: 209 - DNA, 53 bp, synthetic construct
  source 1..53: mol_type = other DNA
  modified_base order(18,24,34): mod_base = OTHER; note = an unnatural base
ggcccgcctgtcgctggnctgaanagtcgctggncaggcgggcccgcgtagcg

SEQ ID NO: 210 - DNA, 43 bp, synthetic construct
  source 1..43: mol_type = other DNA
  modified_base order(26,38): mod_base = OTHER; note = an unnatural base
gcacgctttaacttantggctgggtggnctgggtaaagcgtgc

SEQ ID NO: 211 - DNA, 39 bp, synthetic construct
  source 1..39: mol_type = other DNA
  modified_base order(14,26): mod_base = OTHER; note = an unnatural base
gcgctttaacttantggctgggtggnctgggtaaagcgc

SEQ ID NO: 212 - DNA, 35 bp, synthetic construct
  source 1..35: mol_type = other DNA
  modified_base order(12,24): mod_base = OTHER; note = an unnatural base
gcgttaacttantggctgggtggnctgggtaacgc

SEQ ID NO: 213 - DNA, 34 bp, synthetic construct
  source 1..34: mol_type = other DNA
  modified_base order(10,26): mod_base = OTHER; note = an unnatural base
  modified_base 16: mod_base = OTHER; note = an unnatural base or T
tgtcgctggnctgcanagtcgctggncaagggat

SEQ ID NO: 214 - DNA, 42 bp, synthetic construct
  source 1..42: mol_type = other DNA
  modified_base 2: mod_base = OTHER; note = an unnatural base or T
  modified_base order(16,26,31): mod_base = OTHER; note = an unnatural base
gngtacgcggcgtggntggtgctggntgggncaggcggacaa

SEQ ID NO: 215 - DNA, 42 bp, synthetic construct
  source 1..42: mol_type = other DNA
  modified_base order(12,18,28): mod_base = OTHER; note = an unnatural base or T
ggtgtcgctggnctgganagtcgctggncagaactttagcca

SEQ ID NO: 216 - DNA, 43 bp, synthetic construct
  source 1..43: mol_type = other DNA
  modified_base order(12,18,28): mod_base = OTHER; note = an unnatural base
ggtgtcgctggnctgtanagtcgctggncagtacctttggcca

SEQ ID NO: 217 - DNA, 43 bp, synthetic construct; identical to SEQ ID NO: 216
  source 1..43: mol_type = other DNA
  modified_base order(12,18,28): mod_base = OTHER; note = an unnatural base

SEQ ID NO: 218 - DNA, 45 bp, synthetic construct
  source 1..45: mol_type = other DNA
  modified_base order(12,18,28): mod_base = OTHER; note = an unnatural base
ggtgtcgctggnctgcanagtcgctggncatgaaacctttggccg

SEQ ID NO: 219 - DNA, 42 bp, synthetic construct
  source 1..42: mol_type = other DNA
  modified_base order(12,18,28): mod_base = OTHER; note = an unnatural base
ggagtcgctggnctgtanagtcgctggnctgtagtttaccca

SEQ ID NO: 220 - DNA, 42 bp, synthetic construct; identical to SEQ ID NO: 215
  source 1..42: mol_type = other DNA
  modified_base order(12,18,28): mod_base = OTHER; note = an unnatural base

SEQ ID NO: 221 - DNA, 42 bp, synthetic construct
  source 1..42: mol_type = other DNA
  modified_base order(12,18,28): mod_base = OTHER; note = an unnatural base
cctgtcgctggnctgaanagtcgctggncaggtttccttcgg

SEQ ID NO: 222 - DNA, 42 bp, synthetic construct
  source 1..42: mol_type = other DNA
  modified_base order(12,16,18,28): mod_base = OTHER; note = an unnatural base
cctgtcgctggnctgnanagtcgctggncaggtttccttcgg

SEQ ID NO: 223 - DNA, 42 bp, synthetic construct
  source 1..42: mol_type = other DNA
  modified_base order(12,18,28,34): mod_base = OTHER; note = an unnatural base
cctgtcgctggnctgaanagtcgctggncaggtntccttcgg

SEQ ID NO: 224 - DNA, 42 bp, synthetic construct
  source 1..42: mol_type = other DNA
  modified_base order(12,18,28,38): mod_base = OTHER; note = an unnatural base
cctgtcgctggnctgaanagtcgctggncaggtttccntcgg

SEQ ID NO: 225 - DNA, 42 bp, synthetic construct
  source 1..42: mol_type = other DNA
  modified_base order(12,18,28,34,38): mod_base = OTHER; note = an unnatural base
cctgtcgctggnctgaanagtcgctggncaggtntccntcgg

SEQ ID NO: 226 - DNA, 42 bp, synthetic construct
  source 1..42: mol_type = other DNA
  modified_base order(12,16,18,28,34,38): mod_base = OTHER; note = an unnatural base
cctgtcgctggnctgnanagtcgctggncaggtntccntcgg

SEQ ID NO: 227 - DNA, 40 bp, synthetic construct
  source 1..40: mol_type = other DNA
  modified_base order(12,18,28): mod_base = OTHER; note = an unnatural base
cctgtcgctggnctgaanagtcgctggncaggtttccttc

SEQ ID NO: 228 - DNA, 31 bp, synthetic construct
  source 1..31: mol_type = other DNA
  modified_base order(12,18,28): mod_base = OTHER; note = an unnatural base
cctgtcgctggnctgaanagtcgctggncag

SEQ ID NO: 229 - DNA, 29 bp, synthetic construct
  source 1..29: mol_type = other DNA
  modified_base order(11,17,27): mod_base = OTHER; note = an unnatural base
ctgtcgctggnctgaanagtcgctggnca

SEQ ID NO: 230 - DNA, 29 bp, synthetic construct
  source 1..29: mol_type = other DNA
  modified_base order(11,15,17,27): mod_base = OTHER; note = an unnatural base
ctgtcgctggnctgnanagtcgctggnca

SEQ ID NO: 231 - DNA, 24 bp, synthetic construct
  source 1..24: mol_type = other DNA
  modified_base order(8,14,24): mod_base = OTHER; note = an unnatural base
tcgctggnctgaanagtcgctggn

SEQ ID NO: 232-235 - skipped (4 entries)

SEQ ID NO: 236 - DNA, 67 bp, synthetic construct
  source 1..67: mol_type = other DNA
  modified_base order(20,26,36): mod_base = OTHER; note = an unnatural base
cccggcaaggtgtcgctggnctgganagtcgctggncagaactttagccattgccgggcgcgtagcg

SEQ ID NO: 237 - DNA, 67 bp, synthetic construct
  source 1..67: mol_type = other DNA
  modified_base order(20,26,36): mod_base = OTHER; note = an unnatural base
cccggcgcggtgtcgctggnctgganagtcgctggncagaactttagccagcgccgggcgcgtagcg

SEQ ID NO: 238 - DNA, 67 bp, synthetic construct
  source 1..67: mol_type = other DNA
  modified_base order(20,36): mod_base = OTHER; note = an unnatural base
cttgtcaaggtgtcgctggnctggatagtcgctggncagaactttagccattgacaagcgcgtagcg

SEQ ID NO: 239 - DNA, 10 bp, synthetic construct
  source 1..10: mol_type = other DNA
cccggcaagg

SEQ ID NO: 240 - DNA, 11 bp, synthetic construct
  source 1..11: mol_type = other DNA
ccattgccggg

SEQ ID NO: 241 - DNA, 10 bp, synthetic construct
  source 1..10: mol_type = other DNA
cccggcgcgg

SEQ ID NO: 242 - DNA, 11 bp, synthetic construct
  source 1..11: mol_type = other DNA
ccagcgccggg